European Patent Application EP 4 792 891 A2, published August 19, 2026. Title: MULTISPECIFIC ANTIBODIES AND USES THEREOF. Applicant: LTZ Therapeutics Inc. Application EP, filed July 12, 2024. The sequence listing filed with the application follows.

SEQUENCE LISTING (247 sequences)

SEQ ID NO: 1 - protein, 165 aa, synthetic construct
MNWHMIISGLIVVVLKVVGMTLFLLYFPQIFNKSNDGFTTTRSYGTVCPKDWEFYQARCFFLSTSESSWNESRDFCKGKGSTLAIVNTPEKLKFLQDITDAEKYFIGLIYHREEKRWRWINNSVFNGNVTNQNQNFNCATIGLTKTFDAASCDISYRRICEKNAK

SEQ ID NO: 2 - protein, 190 aa, synthetic construct
MNWHMIISGLIVVVIKVVGMTFFLLYFPQVFGKSNDGFVPTESYGTTSVQNVSQIFGRNDESTMPTRSYGTVCPRNWDFHQGKCFFFSFSESPWKDSMDYCATQGSTLAIVNTPEKLKYLQDIAGIENYFIGLVRQPGEKKWRWINNSVFNGNVTNQDQNFDCVTIGLTKTYDAASCEVSYRWICEMNAK

SEQ ID NO: 3 - protein, 6 aa, synthetic construct
GMYWIC

SEQ ID NO: 4 - protein, 8 aa, synthetic construct
GFSFSGMY

SEQ ID NO: 5 - protein, 17 aa, synthetic construct
CIYTGSSTTGYASWAKG

SEQ ID NO: 6 - protein, 6 aa, synthetic construct
YTGSST

SEQ ID NO: 7 - protein, 13 aa, synthetic construct
PYGDSSHYRGLNL

SEQ ID NO: 8 - protein, 11 aa, synthetic construct
QASQRINNYLS

SEQ ID NO: 9 - protein, 7 aa, synthetic construct
GAATLAS

SEQ ID NO: 10 - protein, 12 aa, synthetic construct
QCTYGIPSSNYG

SEQ ID NO: 11 - protein, 121 aa, synthetic construct
QSLEESGGDLVKPGASLTLTCTASGFSFSGMYWICWVRQAPGKGLEWIACIYTGSSTTGYASWAKGRFTISKTSSTTVTLQMTSLTAADTATHFCASPYGDSSHYRGLNLWGPGTLVTVSS

SEQ ID NO: 12 - protein, 110 aa, synthetic construct
AVVMTQTPASVEAAVGGTVTINCQASQRINNYLSWFQQKPGQPPKLLIYGAATLASGVPSRFKGSGSGTEYTLTISDLEPADAATYYCQCTYGIPSSNYGFGGGTEVVVK

SEQ ID NO: 13 - protein, 6 aa, synthetic construct
RSSYMC

SEQ ID NO: 14 - protein, 8 aa, synthetic construct
GFSFSRSS

SEQ ID NO: 15 - protein, 17 aa, synthetic construct
CLSVGDGHTYYASWAKG

SEQ ID NO: 16 - protein, 6 aa, synthetic construct
SVGDGH

SEQ ID NO: 17 - protein, 14 aa, synthetic construct
APSYSGDGGHGYDL

SEQ ID NO: 18 - protein, 13 aa, synthetic construct
QASESVDRNNRLA

SEQ ID NO: 19 - protein, 7 aa, synthetic construct
TTSTLAS

SEQ ID NO: 20 - protein, 12 aa, synthetic construct
AGYRGAHTDGDA

SEQ ID NO: 21 - protein, 122 aa, synthetic construct
QSLEESGGDLVKPGASLTLTCTASGFSFSRSSYMCWVRQAPGKGLEWIGCLSVGDGHTYYASWAKGRFTISKTSSTSVTLQMTRLTAADTATYFCARAPSYSGDGGHGYDLWGPGTLVTVSS

SEQ ID NO: 22 - protein, 112 aa, synthetic construct
AIVMTQTPSSKSVPVGDTVTINCQASESVDRNNRLAWFQQKPGQPPKLLIYTTSTLASGVPSRFKGSGSGTHFTLTISDVVPDDAATYYCAGYRGAHTDGDAFGGGTEVVVK

SEQ ID NO: 23 - protein, 6 aa, synthetic construct
SSYYMC

SEQ ID NO: 24 - protein, 8 aa, synthetic construct
GFSFSSSY

SEQ ID NO: 25 - protein, 17 aa, synthetic construct
CIYSSSGRTWYATWVNG

SEQ ID NO: 26 - protein, 6 aa, synthetic construct
YSSSGR

SEQ ID NO: 27 - protein, 15 aa, synthetic construct
SYAGYGGYGYAYFNL

SEQ ID NO: 28 - protein, 11 aa, synthetic construct
QASEDIYSSLA

SEQ ID NO: 29 - protein, 7 aa, synthetic construct
DASTLAS

SEQ ID NO: 30 - protein, 14 aa, synthetic construct
QNYYDSTGSGYGAA

SEQ ID NO: 31 - protein, 125 aa, synthetic construct
QQQLEESGGGLVKPGGTLTLTCTASGFSFSSSYYMCWVRQAPGKGLELIACIYSSSGRTWYATWVNGRFTISRSTSLNTVDLKMTSLTAADTATYFCARSYAGYGGYGYAYFNLWGPGTLVTVSS

SEQ ID NO: 32 - protein, 112 aa, synthetic construct
DIVMTQTPASVEAGVGGTVTIKCQASEDIYSSLAWYQQKAGQRPKLLIYDASTLASGVPSRFKGSGSGTEYTLTISGVQPDDAATYYCQNYYDSTGSGYGAAFGGGTEVVVK

SEQ ID NO: 33 - protein, 6 aa, synthetic construct
SNKYMC

SEQ ID NO: 34 - protein, 8 aa, synthetic construct
GFSFTSNK

SEQ ID NO: 35 - protein, 17 aa, synthetic construct
CIYVGDGNTYYASWAKG

SEQ ID NO: 36 - protein, 6 aa, synthetic construct
YVGDGN

SEQ ID NO: 37 - protein, 15 aa, synthetic construct
GGDYSIGGGGFASNL

SEQ ID NO: 38 - protein, 11 aa, synthetic construct
QASESISNFLA

SEQ ID NO: 39 - protein, 7 aa, synthetic construct
RASTLAS

SEQ ID NO: 40 - protein, 13 aa, synthetic construct
QSYYGTSSTGHNV

SEQ ID NO: 41 - protein, 123 aa, synthetic construct
QSLEESGGDLVKPGASLTLTCTASGFSFTSNKYMCWVRQAPGKGPEWIACIYVGDGNTYYASWAKGRFTISKTSSTTVTLQMTSLTVADTATYFCARGGDYSIGGGGFASNLWGPGTLVTVSS

SEQ ID NO: 42 - protein, 111 aa, synthetic construct
AFELTQTPSSVEAAVGGTVTINCQASESISNFLAWYRQKPGQPPKLLIYRASTLASGVSSRFKGSGSGTEFTLTISDLEPADGASYYCQSYYGTSSTGHNVFGGGTEVVVK

SEQ ID NO: 43 - protein, 6 aa, synthetic construct
SGYDMC

SEQ ID NO: 44 - protein, 8 aa, synthetic construct
GFSFSSGY

SEQ ID NO: 45 - protein, 18 aa, synthetic construct
CIYGGRSDNVYYARWAKG

SEQ ID NO: 46 - protein, 7 aa, synthetic construct
YGGRSDN

SEQ ID NO: 47 - protein, 17 aa, synthetic construct
DYLYRGYIGGGYGRSNL

SEQ ID NO: 48 - protein, 11 aa, synthetic construct
RASEDIENCLA

SEQ ID NO: 49 - protein, 7 aa, synthetic construct
QASKLPS

SEQ ID NO: 50 - protein, 12 aa, synthetic construct
QNPDYMRNTDNL

SEQ ID NO: 51 - protein, 127 aa, synthetic construct
QQQLEESGGGLVKPGGTLTLTCKASGFSFSSGYDMCWVRQAPGKGLEWIACIYGGRSDNVYYARWAKGRFTISKTSSTTVTLQMTSLTAADTATYFCARDYLYRGYIGGGYGRSNLWGPGTLVTVSS

SEQ ID NO: 52 - protein, 110 aa, synthetic construct
DVVMTQTPASVSAAVGGTVTINCRASEDIENCLAWYQQKPGQPPKLLIYQASKLPSGVPSRFSGSGSGTEYTLTISDLEPDDGATYYCQNPDYMRNTDNLFGGGTEVVVK

SEQ ID NO: 53 - protein, 6 aa, synthetic construct
NYYYMC

SEQ ID NO: 54 - protein, 8 aa, synthetic construct
GFDLNNYY

SEQ ID NO: 55 - protein, 18 aa, synthetic construct
CTHAGSSSSSYYARWAKG

SEQ ID NO: 56 - protein, 7 aa, synthetic construct
HAGSSSS

SEQ ID NO: 57 - protein, 10 aa, synthetic construct
HDRDYDDMDL

SEQ ID NO: 58 - protein, 12 aa, synthetic construct
QASQSIEYGYLS

SEQ ID NO: 59 - protein, 7 aa, synthetic construct
YASKLAS

SEQ ID NO: 60 - protein, 12 aa, synthetic construct
LYGYFDDYSGAA

SEQ ID NO: 61 - protein, 119 aa, synthetic construct
QSLEESGGGLVQPEGSLTLTCTASGFDLNNYYYMCWVRQAPGKGLEWIACTHAGSSSSSYYARWAKGRFTISKTSSTTVTLQMTSLTAADTATYFCARHDRDYDDMDLWGPGTLVTVSS

SEQ ID NO: 62 - protein, 111 aa, synthetic construct
NIVMTQTTSPVSAVVGGTITINCQASQSIEYGYLSWYQQKPGQPPKLLIFYASKLASGVPSRFSGSGSGTQFTLTISGVQPDDAATYFCLYGYFDDYSGAAFGGGTEVVVK

SEQ ID NO: 63 - protein, 6 aa, synthetic construct
SSYWLC

SEQ ID NO: 64 - protein, 8 aa, synthetic construct
GFSFSSSY

SEQ ID NO: 65 - protein, 18 aa, synthetic construct
CIYGGSSRGTYYASWAKG

SEQ ID NO: 66 - protein, 7 aa, synthetic construct
YGGSSRG

SEQ ID NO: 67 - protein, 14 aa, synthetic construct
HTYTYPRFSPYFNL

SEQ ID NO: 68 - protein, 11 aa, synthetic construct
QASEDIESSLA

SEQ ID NO: 69 - protein, 7 aa, synthetic construct
DASDLES

SEQ ID NO: 70 - protein, 12 aa, synthetic construct
QSAYYTGSADNT

SEQ ID NO: 71 - protein, 123 aa, synthetic construct
QSLEESGGDLVKPGGTLTLTCTASGFSFSSSYWLCWVRQAPGKGLEWIACIYGGSSRGTYYASWAKGRFTISKTSSTTVTLQMTSLTAADTATYFCASHTYTYPRFSPYFNLWGPGTLVSVSS

SEQ ID NO: 72 - protein, 110 aa, synthetic construct
AFEMTQTPASVSPAVGGTVSINCQASEDIESSLAWYQQKPGQPPKLLIYDASDLESGVPSRFKGSGSGTEYTLTISGVQPADAATYFCQSAYYTGSADNTFGGGTEVVVK

SEQ ID NO: 73 - protein, 6 aa, synthetic construct
SYYYMC

SEQ ID NO: 74 - protein, 8 aa, synthetic construct
GFTLSSYY

SEQ ID NO: 75 - protein, 18 aa, synthetic construct
CIYAGSSGTTVYASWAKG

SEQ ID NO: 76 - protein, 7 aa, synthetic construct
YAGSSGT

SEQ ID NO: 77 - protein, 15 aa, synthetic construct
KLGDVGYGHTTYFNL

SEQ ID NO: 78 - protein, 11 aa, synthetic construct
QASQNIYSTLA

SEQ ID NO: 79 - protein, 7 aa, synthetic construct
DASDLAS

SEQ ID NO: 80 - protein, 13 aa, synthetic construct
QTYYDSGSDDLNA

SEQ ID NO: 81 - protein, 124 aa, synthetic construct
QSLEESGGGLVKPEGSLTLTCKASGFTLSSYYYMCWVRQAPGKGLEWIACIYAGSSGTTVYASWAKGRFTISKTSSTTVTLQMTSLTAADTATYLCARKLGDVGYGHTTYFNLWGPGTLVTVSS

SEQ ID NO: 82 - protein, 111 aa, synthetic construct
ALVMTQTPSSVSAAVGGTVTIKCQASQNIYSTLAWYQQKPGQPPKLLMFDASDLASGVPSRFKGSGSGTEYTLTISDLEPADAATYFCQTYYDSGSDDLNAFGGGTEVVVK

SEQ ID NO: 83 - protein, 123 aa, synthetic construct
EQQLLESGGGLVQPGGSLRLSCAASGFSFSGMYWICWVRQAPGKGLEWIACIYTGSSTTGYASWAKGRFTISKDSSKNTVYLQMNSLRAEDTAVYFCASPYGDSSHYRGLNLWGPGTLVTVSS

SEQ ID NO: 84 - protein, 110 aa, synthetic construct
DVQMTQSPSSLSASVGDRVTITCQASQRINNYLSWFQQKPGKPPKLLIYGAATLASGVPSRFSGSGSGTDYTLTISSLQPEDVATYYCQCTYGIPSSNYGFGGGTKVEIK

SEQ ID NO: 85 - protein, 124 aa, synthetic construct
EQQLVESGGGLVKPGGSLRLSCAASGFSFSRSSYMCWVRQAPGKCLEWIGCLSVGDGHTYYASWAKGRFTISKDSAKNSVYLQMNSLRAEDTAVYFCARAPSYSGDGGHGYDLWGPGTLVTVSS

SEQ ID NO: 86 - protein, 112 aa, synthetic construct
DIQMTQSPSSLSASVGDRVTITCQASESVDRNNRLAWFQQKPGKPPKLLIYTTSTLASGVPSRFSGSGSGTDFTLTISSLQPEDVATYYCAGYRGAHTDGDAFGCGTKVEIK

SEQ ID NO: 87 - protein, 125 aa, synthetic construct
EQQLVESGGGLVQPGGSLRLSCSASGFSFSSSYYMCWVRQAPGKGLELIACIYSSSGRTWYATWVNGRFTISRDTSKNTVYLQMNSLRAEDTAVYFCARSYAGYGGYGYAYFNLWGPGTLVTVSS

SEQ ID NO: 88 - protein, 112 aa, synthetic construct
EIVMTQSPATLSVSPGERATLSCQASEDIYSSLAWYQQKPGQRPRLLIYDASTLASGVPARFSGSGSGTEYTLTISSLQSEDFAVYYCQNYYDSTGSGYGAAFGGGTKVEIK

SEQ ID NO: 89 - protein, 128 aa, synthetic construct
EQQLVESGGGVVQPGRSLRLSCAASGFSFSSGYDMCWVRQAPGKGLEWIACIYGGRSDNVYYARWAKGRFTISKDSSTNTVFLQMNSLRAEDTAVYFCARDYLYRGYIGGGYGRSNLWGPGTLVTVSS

SEQ ID NO: 90 - protein, 110 aa, synthetic construct
DVQMTQSPSSVSASVGDRVTITCRASEDIENCLAWYQQKPGKPPKLLIYQASKLPSGVPSRFSGSGSGTDYTLTISSLQPEDFATYYCQNPDYMRNTDNLFGGGTKVEIK

SEQ ID NO: 91 - protein, 125 aa, synthetic construct
EQQLLESGGGLVQPGGSLRLSCAASGFSFSSSYWLCWVRQAPGKGLEWIACIYGGSSRGTYYASWAKGRFTISKDSSKNTVYLQMNSLRAEDTAVYFCASHTYTYPRFSPYFNLWGPGTLVTVSS

SEQ ID NO: 92 - protein, 110 aa, synthetic construct
EFVMTQSPATLSVSPGERATLSCQASEDIESSLAWYQQKPGQPPRLLIYDASDLESGVPARFSGSGSGTEYTLTISSLQSEDFAVYFCQSAYYTGSADNTFGGGTKVEIK

SEQ ID NO: 93 - protein, 121 aa, synthetic construct
QIQLVQSGPELKKPGETVKISCKASGYTFTIYAMNWVKQAPGKGLEWMGWINTDTGEPTYADDFKGRFAFSLETSASTAYLQINNLKNEDMATYFCARSSEVFYDYRFDYWGQGTALTVSS

SEQ ID NO: 94 - protein, 108 aa, synthetic construct
DIQMTQSPSSLSASLGERVSLTCRASQDIGSSLNWLQQEPDGTIKRLIYATSNLDSGVPKRFSGSRSGSDYSLTISSLESEDFVHYYCLQYASSPFTFGSGTKLEIKR

SEQ ID NO: 95 - protein, 330 aa, synthetic construct [sequence omitted]

SEQ ID NO: 96 - protein, 330 aa, synthetic construct
ASTKGPSVFPLAPSSKSTSGGTAALGCLVKDYFPEPVTVSWNSGALTSGVHTFPAVLQSSGLYSLSSVVTVPSSSLGTQTYICNVNHKPSNTKVDKKVEPKSCDKTHTCPPCPAPEAAGGPSVFLFPPKPKDTLMISRTPEVTCVVVDVSHEDPEVKFNWYVDGVEVHNAKTKPREEQYNSTYRVVSVLTVLHQDWLNGKEYKCKVSNKALGAPIEKTISKAKGQPREPQVYTLPPSRDELTKNQVSLTCLVKGFYPSDIAVEWESNGQPENNYKTTPPVLDSDGSFFLYSKLTVDKSRWQQGNVFSCSVMHEALHNHYTQKSLSLSPGK

SEQ ID NO: 97 - protein, 330 aa, synthetic construct
ASTKGPSVFPLAPSSKSTSGGTAALGCLVKDYFPEPVTVSWNSGALTSGVHTFPAVLQSSGLYSLSSVVTVPSSSLGTQTYICNVNHKPSNTKVDKKVEPKSCDKTHTCPPCPAPELLAGPSVFLFPPKPKDTLMISRTPEVTCVVVDVSHEDPEVKFNWYVDGVEVHNAKTKPREEQYNSTYRVVSVLTVLHQDWLNGKEYKCKVSNKALPLPEEKTISKAKGQPREPQVYTLPPSRDELTKNQVSLTCLVKGFYPSDIAVEWESNGQPENNYKTTPPVLDSDGSFFLYSKLTVDKSRWQQGNVFSCSVMHEALHNHYTQKSLSLSPGK

SEQ ID NO: 98 - protein, 107 aa, synthetic construct [sequence omitted]

SEQ ID NO: 99 - protein, 5 aa, synthetic construct
GGGGS

SEQ ID NO: 100 - protein, 5 aa, synthetic construct
DTYIH

SEQ ID NO: 101 - protein, 7 aa, synthetic construct
GFNIKDT

SEQ ID NO: 102 - protein, 17 aa, synthetic construct
RIYPTNGYTRYADSVKG

SEQ ID NO: 103 - protein, 6 aa, synthetic construct
YPTNGY

SEQ ID NO: 104 - protein, 11 aa, synthetic construct
WGGDGFYAMDY

SEQ ID NO: 105 - protein, 11 aa, synthetic construct
RASQDVNTAVA

SEQ ID NO: 106 - protein, 7 aa, synthetic construct
SASFLYS

SEQ ID NO: 107 - protein, 9 aa, synthetic construct
QQHYTTPPT

SEQ ID NO: 108 - protein, 120 aa, synthetic construct [sequence omitted]

SEQ ID NO: 109 - protein, 107 aa, synthetic construct [sequence omitted]

SEQ ID NO: 110 - protein, 450 aa, synthetic construct
EVQLVESGGGLVQPGGSLRLSCAASGFNIKDTYIHWVRQAPGKGLEWVARIYPTNGYTRYADSVKGRFTISADTSKNTAYLQMNSLRAEDTAVYYCSRWGGDGFYAMDYWGQGTLVTVSSASTKGPSVFPLAPSSKSTSGGTAALGCLVKDYFPEPVTVSWNSGALTSGVHTFPAVLQSSGLYSLSSVVTVPSSSLGTQTYICNVNHKPSNTKVDKKVEPKSCDKTHTCPPCPAPEAAGGPSVFLFPPKPKDTLMISRTPEVTCVVVDVSHEDPEVKFNWYVDGVEVHNAKTKPREEQYNSTYRVVSVLTVLHQDWLNGKEYKCKVSNKALGAPIEKTISKAKGQPREPQVCTLPPSRDELTKNQVSLSCAVKGFYPSDIAVEWESNGQPENNYKTTPPVLDSDGSFFLVSKLTVDKSRWQQGNVFSCSVMHEALHNRFTQKSLSLSPGK

SEQ ID NO: 111 - protein, 455 aa, synthetic construct
QSLEESGGDLVKPGASLTLTCTASGFSFSGMYWICWVRQAPGKGLEWIACIYTGSSTTGYASWAKGRFTISKTSSTTVTLQMTSLTAADTATHFCASPYGDSSHYRGLNLWGPGTLVTVSSRTVAAPSVFIFPPSDEQLKSGTASVVCLLNNFYPREAKVQWKVDNALQSGNSQESVTEQDSKDSTYSLSSTLTLSKADYEKHKVYACEVTHQGLSSPVTKSFNRGECDKTHTCPPCPAPEAAGGPSVFLFPPKPKDTLMISRTPEVTCVVVDVSHEDPEVKFNWYVDGVEVHNAKTKPREEQYNSTYRVVSVLTVLHQDWLNGKEYKCKVSNKALGAPIEKTISKAKGQPREPQVYTLPPCRDELTKNQVSLWCLVKGFYPSDIAVEWESNGQPENNYKTTPPVLDSDGSFFLYSKLTVDKSRWQQGNVFSCSVMHEALHNHYTQKSLSLSPGK

SEQ ID NO: 112 - protein, 214 aa, synthetic construct
DIQMTQSPSSLSASVGDRVTITCRASQDVNTAVAWYQQKPGKAPKLLIYSASFLYSGVPSRFSGSRSGTDFTLTISSLQPEDFATYYCQQHYTTPPTFGQGTKVEIKRTVAAPSVFIFPPSDEQLKSGTASVVCLLNNFYPREAKVQWKVDNALQSGNSQESVTEQDSKDSTYSLSSTLTLSKADYEKHKVYACEVTHQGLSSPVTKSFNRGEC

SEQ ID NO: 113 - protein, 215 aa, synthetic construct
AVVMTQTPASVEAAVGGTVTINCQASQRINNYLSWFQQKPGQPPKLLIYGAATLASGVPSRFKGSGSGTEYTLTISDLEPADAATYYCQCTYGIPSSNYGFGGGTEVVVKSSASTKGPSVFPLAPSSKSTSGGTAALGCLVKDYFPEPVTVSWNSGALTSGVHTFPAVLQSSGLYSLSSVVTVPSSSLGTQTYICNVNHKPSNTKVDKKVEPKSC

SEQ ID NO: 114 - protein, 450 aa, synthetic construct; identical to SEQ ID NO: 110

SEQ ID NO: 115 - protein, 456 aa, synthetic construct
QSLEESGGDLVKPGASLTLTCTASGFSFSRSSYMCWVRQAPGKGLEWIGCLSVGDGHTYYASWAKGRFTISKTSSTSVTLQMTRLTAADTATYFCARAPSYSGDGGHGYDLWGPGTLVTVSSRTVAAPSVFIFPPSDEQLKSGTASVVCLLNNFYPREAKVQWKVDNALQSGNSQESVTEQDSKDSTYSLSSTLTLSKADYEKHKVYACEVTHQGLSSPVTKSFNRGECDKTHTCPPCPAPEAAGGPSVFLFPPKPKDTLMISRTPEVTCVVVDVSHEDPEVKFNWYVDGVEVHNAKTKPREEQYNSTYRVVSVLTVLHQDWLNGKEYKCKVSNKALGAPIEKTISKAKGQPREPQVYTLPPCRDELTKNQVSLWCLVKGFYPSDIAVEWESNGQPENNYKTTPPVLDSDGSFFLYSKLTVDKSRWQQGNVFSCSVMHEALHNHYTQKSLSLSPGK

SEQ ID NO: 116 - protein, 214 aa, synthetic construct; identical to SEQ ID NO: 112

SEQ ID NO: 117 - protein, 217 aa, synthetic construct
AIVMTQTPSSKSVPVGDTVTINCQASESVDRNNRLAWFQQKPGQPPKLLIYTTSTLASGVPSRFKGSGSGTHFTLTISDVVPDDAATYYCAGYRGAHTDGDAFGGGTEVVVKSSASTKGPSVFPLAPSSKSTSGGTAALGCLVKDYFPEPVTVSWNSGALTSGVHTFPAVLQSSGLYSLSSVVTVPSSSLGTQTYICNVNHKPSNTKVDKKVEPKSC

SEQ ID NO: 118 - protein, 450 aa, synthetic construct
EVQLVESGGGLVQPGGSLRLSCAASGFNIKDTYIHWVRQAPGKGLEWVARIYPTNGYTRYADSVKGRFTISADTSKNTAYLQMNSLRAEDTAVYYCSRWGGDGFYAMDYWGQGTLVTVSSASTKGPSVFPLAPSSKSTSGGTAALGCLVKDYFPEPVTVSWNSGALTSGVHTFPAVLQSSGLYSLSSVVTVPSSSLGTQTYICNVNHKPSNTKVDKKVEPKSCDKTHTCPPCPAPEAAGGPSVFLFPPKPKDTLMISRTPEVTCVVVDVSHEDPEVKFNWYVDGVEVHNAKTKPREEQYNSTYRVVSVLTVLHQDWLNGKEYKCKVSNKALGAPIEKTISKAKGQPREPQVYTLPPSRDELTKNQVSLTCLVKGFYPSDIAVEWESNGQPENNYKTTPPVLDSDGSFFLYSKLTVDKSRWQQGNVFSCSVMHEALHNHYTQKSLSLSPGK

SEQ ID NO: 119 - protein, 480 aa, synthetic construct
DIQMTQSPSSLSASVGDRVTITCRASQDVNTAVAWYQQKPGKAPKLLIYSASFLYSGVPSRFSGSRSGTDFTLTISSLQPEDFATYYCQQHYTTPPTFGQGTKVEIKRTVAAPSVFIFPPSDEQLKSGTASVVCLLNNFYPREAKVQWKVDNALQSGNSQESVTEQDSKDSTYSLSSTLTLSKADYEKHKVYACEVTHQGLSSPVTKSFNRGECGGGGSGGGGSGGGGSAVVMTQTPASVEAAVGGTVTINCQASQRINNYLSWFQQKPGQPPKLLIYGAATLASGVPSRFKGSGSGTEYTLTISDLEPADAATYYCQCTYGIPSSNYGFGGGTEVVVKGGGGSGGGGSGGGGSGGGGSQSLEESGGDLVKPGASLTLTCTASGFSFSGMYWICWVRQAPGKGLEWIACIYTGSSTTGYASWAKGRFTISKTSSTTVTLQMTSLTAADTATHFCASPYGDSSHYRGLNLWGPGTLVTVSS

SEQ ID NO: 120 - protein, 450 aa, synthetic construct; identical to SEQ ID NO: 118

SEQ ID NO: 121 - protein, 483 aa, synthetic construct
DIQMTQSPSSLSASVGDRVTITCRASQDVNTAVAWYQQKPGKAPKLLIYSASFLYSGVPSRFSGSRSGTDFTLTISSLQPEDFATYYCQQHYTTPPTFGQGTKVEIKRTVAAPSVFIFPPSDEQLKSGTASVVCLLNNFYPREAKVQWKVDNALQSGNSQESVTEQDSKDSTYSLSSTLTLSKADYEKHKVYACEVTHQGLSSPVTKSFNRGECGGGGSGGGGSGGGGSAIVMTQTPSSKSVPVGDTVTINCQASESVDRNNRLAWFQQKPGQPPKLLIYTTSTLASGVPSRFKGSGSGTHFTLTISDVVPDDAATYYCAGYRGAHTDGDAFGGGTEVVVKGGGGSGGGGSGGGGSGGGGSQSLEESGGDLVKPGASLTLTCTASGFSFSRSSYMCWVRQAPGKGLEWIGCLSVGDGHTYYASWAKGRFTISKTSSTSVTLQMTRLTAADTATYFCARAPSYSGDGGHGYDLWGPGTLVTVSS

SEQ ID NO: 122 - protein, 450 aa, synthetic construct
EVQLVESGGGLVQPGGSLRLSCAASGFNIKDTYIHWVRQAPGKGLEWVARIYPTNGYTRYADSVKGRFTISADTSKNTAYLQMNSLRAEDTAVYYCSRWGGDGFYAMDYWGQGTLVTVSSASTKGPSVFPLAPSSKSTSGGTAALGCLVKDYFPEPVTVSWNSGALTSGVHTFPAVLQSSGLYSLSSVVTVPSSSLGTQTYICNVNHKPSNTKVDKKVEPKSCDKTHTCPPCPAPELLAGPSVFLFPPKPKDTLMISRTPEVTCVVVDVSHEDPEVKFNWYVDGVEVHNAKTKPREEQYNSTYRVVSVLTVLHQDWLNGKEYKCKVSNKALPLPEEKTISKAKGQPREPQVYTLPPSRDELTKNQVSLTCLVKGFYPSDIAVEWESNGQPENNYKTTPPVLDSDGSFFLYSKLTVDKSRWQQGNVFSCSVMHEALHNHYTQKSLSLSPGK

SEQ ID NO: 123 - protein, 483 aa, synthetic construct
DIQMTQSPSSLSASVGDRVTITCRASQDVNTAVAWYQQKPGKAPKLLIYSASFLYSGVPSRFSGSRSGTDFTLTISSLQPEDFATYYCQQHYTTPPTFGQGTKVEIKRTVAAPSVFIFPPSDEQLKSGTASVVCLLNNFYPREAKVQWKVDNALQSGNSQESVTEQDSKDSTYSLSSTLTLSKADYEKHKVYACEVTHQGLSSPVTKSFNRGECGGGGSGGGGSGGGGSAIVMTQTPSSKSVPVGDTVTINCQASESVDRNNRLAWFQQKPGQPPKLLIYTTSTLASGVPSRFKGSGSGTHFTLTISDVVPDDAATYYCAGYRGAHTDGDAFGCGTEVVVKGGGGSGGGGSGGGGSGGGGSQSLEESGGDLVKPGASLTLTCTASGFSFSRSSYMCWVRQAPGKCLEWIGCLSVGDGHTYYASWAKGRFTISKTSSTSVTLQMTRLTAADTATYFCARAPSYSGDGGHGYDLWGPGTLVTVSS

SEQ ID NO: 124 - protein, 450 aa, synthetic construct; identical to SEQ ID NO: 118

SEQ ID NO: 125 - protein, 214 aa, synthetic construct; identical to SEQ ID NO: 112

SEQ ID NO: 126 - protein, 5 aa, synthetic construct
TYGMH

SEQ ID NO: 127 - protein, 7 aa, synthetic construct
GFTFSTY

SEQ ID NO: 128 - protein, 17 aa, synthetic construct
VIWDDGSYKYYGDSVKG

SEQ ID NO: 129 - protein, 6 aa, synthetic construct
WDDGSY

SEQ ID NO: 130 - protein, 16 aa, synthetic construct
DGITMVRGVMKDYFDY

SEQ ID NO: 131 - protein, 11 aa, synthetic construct
RASQDISSALV

SEQ ID NO: 132 - protein, 7 aa, synthetic construct
DASSLES

SEQ ID NO: 133 - protein, 9 aa, synthetic construct
QQFNSYPLT

SEQ ID NO: 134 - protein, 125 aa, synthetic construct [sequence omitted]

SEQ ID NO: 135 - protein, 107 aa, synthetic construct [sequence omitted]

SEQ ID NO: 136 - protein, 5 aa, synthetic construct
NYYIY

SEQ ID NO: 137 - protein, 7 aa, synthetic construct
GYTFTNY

SEQ ID NO: 138 - protein, 17 aa, synthetic construct
GINPTSGGSNFNEKFKT

SEQ ID NO: 139 - protein, 6 aa, synthetic construct
NPTSGG

SEQ ID NO: 140 - protein, 14 aa, synthetic construct
QGLWFDSDGRGFDF

SEQ ID NO: 141 - protein, 16 aa, synthetic construct
RSSQNIVHSNGNTYLD

SEQ ID NO: 142 - protein, 7 aa, synthetic construct
KVSNRFS

SEQ ID NO: 143 - protein, 9 aa, synthetic construct
FQYSHVPWT

SEQ ID NO: 144 - protein, 123 aa, synthetic construct [sequence omitted]

SEQ ID NO: 145 - protein, 112 aa, synthetic construct
DIQMTQSPSSLSASVGDRVTITCRSSQNIVHSNGNTYLDWYQQTPGKAPKLLIYKVSNRFSGVPSRFSGSGSGTDFTFTISSLQPEDIATYYCFQYSHVPWTFGQGTKLEIK

SEQ ID NO: 146 - protein, 455 aa, synthetic construct
QVQLVESGGGVVQPGRSLRLSCAASGFTFSTYGMHWVRQAPGKGLEWVAVIWDDGSYKYYGDSVKGRFTISRDNSKNTLYLQMNSLRAEDTAVYYCARDGITMVRGVMKDYFDYWGQGTLVTVSSASTKGPSVFPLAPSSKSTSGGTAALGCLVKDYFPEPVTVSWNSGALTSGVHTFPAVLQSSGLYSLSSVVTVPSSSLGTQTYICNVNHKPSNTKVDKKVEPKSCDKTHTCPPCPAPELLAGPSVFLFPPKPKDTLMISRTPEVTCVVVDVSHEDPEVKFNWYVDGVEVHNAKTKPREEQYNSTYRVVSVLTVLHQDWLNGKEYKCKVSNKALPLPEEKTISKAKGQPREPQVYTLPPSRDELTKNQVSLTCLVKGFYPSDIAVEWESNGQPENNYKTTPPVLDSDGSFFLYSKLTVDKSRWQQGNVFSCSVMHEALHNHYTQKSLSLSPGK

SEQ ID NO: 147 - protein, 483 aa, synthetic construct
AIQLTQSPSSLSASVGDRVTITCRASQDISSALVWYQQKPGKAPKLLIYDASSLESGVPSRFSGSESGTDFTLTISSLQPEDFATYYCQQFNSYPLTFGGGTKVEIKRTVAAPSVFIFPPSDEQLKSGTASVVCLLNNFYPREAKVQWKVDNALQSGNSQESVTEQDSKDSTYSLSSTLTLSKADYEKHKVYACEVTHQGLSSPVTKSFNRGECGGGGSGGGGSGGGGSAIVMTQTPSSKSVPVGDTVTINCQASESVDRNNRLAWFQQKPGQPPKLLIYTTSTLASGVPSRFKGSGSGTHFTLTISDVVPDDAATYYCAGYRGAHTDGDAFGCGTEVVVKGGGGSGGGGSGGGGSGGGGSQSLEESGGDLVKPGASLTLTCTASGFSFSRSSYMCWVRQAPGKCLEWIGCLSVGDGHTYYASWAKGRFTISKTSSTSVTLQMTRLTAADTATYFCARAPSYSGDGGHGYDLWGPGTLVTVSS

SEQ ID NO: 148 - protein, 453 aa, synthetic construct
QVQLQQSGAEVKKPGSSVKVSCKASGYTFTNYYIYWVRQAPGQGLEWIGGINPTSGGSNFNEKFKTRVTITADESSTTAYMELSSLRSEDTAFYFCTRQGLWFDSDGRGFDFWGQGTTVTVSSASTKGPSVFPLAPSSKSTSGGTAALGCLVKDYFPEPVTVSWNSGALTSGVHTFPAVLQSSGLYSLSSVVTVPSSSLGTQTYICNVNHKPSNTKVDKKVEPKSCDKTHTCPPCPAPELLAGPSVFLFPPKPKDTLMISRTPEVTCVVVDVSHEDPEVKFNWYVDGVEVHNAKTKPREEQYNSTYRVVSVLTVLHQDWLNGKEYKCKVSNKALPLPEEKTISKAKGQPREPQVYTLPPSRDELTKNQVSLTCLVKGFYPSDIAVEWESNGQPENNYKTTPPVLDSDGSFFLYSKLTVDKSRWQQGNVFSCSVMHEALHNHYTQKSLSLSPGK

SEQ ID NO: 149 - protein, 488 aa, synthetic construct
DIQMTQSPSSLSASVGDRVTITCRSSQNIVHSNGNTYLDWYQQTPGKAPKLLIYKVSNRFSGVPSRFSGSGSGTDFTFTISSLQPEDIATYYCFQYSHVPWTFGQGTKLEIKRTVAAPSVFIFPPSDEQLKSGTASVVCLLNNFYPREAKVQWKVDNALQSGNSQESVTEQDSKDSTYSLSSTLTLSKADYEKHKVYACEVTHQGLSSPVTKSFNRGECGGGGSGGGGSGGGGSAIVMTQTPSSKSVPVGDTVTINCQASESVDRNNRLAWFQQKPGQPPKLLIYTTSTLASGVPSRFKGSGSGTHFTLTISDVVPDDAATYYCAGYRGAHTDGDAFGCGTEVVVKGGGGSGGGGSGGGGSGGGGSQSLEESGGDLVKPGASLTLTCTASGFSFSRSSYMCWVRQAPGKCLEWIGCLSVGDGHTYYASWAKGRFTISKTSSTSVTLQMTRLTAADTATYFCARAPSYSGDGGHGYDLWGPGTLVTVSS

SEQ ID NO: 150 - protein, 5 aa, synthetic construct
NYLIE

SEQ ID NO: 151 - protein, 7 aa, synthetic construct
GYAFTNY

SEQ ID NO: 152 - protein, 17 aa, synthetic construct
VINPGSGGTNYNEKFKG

SEQ ID NO: 153 - protein, 6 aa, synthetic construct
NPGSGG

SEQ ID NO: 154 - protein, 7 aa, synthetic construct
DGPWFAY

SEQ ID NO: 155 - protein, 11 aa, synthetic construct
KASENVVTYVS

SEQ ID NO: 156 - protein, 7 aa, synthetic construct
GASNRYT

SEQ ID NO: 157 - protein, 9 aa, synthetic construct
GQGYSYPYT

SEQ ID NO: 158 - protein, 116 aa, synthetic construct
QVQLQQSGAELVRPGTSVKVSCKASGYAFTNYLIEWVKQRPGQGLEWIGVINPGSGGTNYNEKFKGKATLTADKSSSTAYMQLSSLTSDDSAVYFCARDGPWFAYWGQGTLVTVSA

SEQ ID NO: 159 - protein, 107 aa, synthetic construct
NIVMTQSPKSMSMSVGERVTLTCKASENVVTYVSWYQQKPEQSPKLLIYGASNRYTGVPDRFTGSGSATDFTLTISSVQAEDLADYHCGQGYSYPYTFGGGTKLEIK

SEQ ID NO: 160 - protein, 446 aa, synthetic construct
QVQLQQSGAELVRPGTSVKVSCKASGYAFTNYLIEWVKQRPGQGLEWIGVINPGSGGTNYNEKFKGKATLTADKSSSTAYMQLSSLTSDDSAVYFCARDGPWFAYWGQGTLVTVSAASTKGPSVFPLAPSSKSTSGGTAALGCLVKDYFPEPVTVSWNSGALTSGVHTFPAVLQSSGLYSLSSVVTVPSSSLGTQTYICNVNHKPSNTKVDKKVEPKSCDKTHTCPPCPAPELLAGPSVFLFPPKPKDTLMISRTPEVTCVVVDVSHEDPEVKFNWYVDGVEVHNAKTKPREEQYNSTYRVVSVLTVLHQDWLNGKEYKCKVSNKALPLPEEKTISKAKGQPREPQVYTLPPSRDELTKNQVSLTCLVKGFYPSDIAVEWESNGQPENNYKTTPPVLDSDGSFFLYSKLTVDKSRWQQGNVFSCSVMHEALHNHYTQKSLSLSPGK

SEQ ID NO: 161 - protein, 483 aa, synthetic construct
NIVMTQSPKSMSMSVGERVTLTCKASENVVTYVSWYQQKPEQSPKLLIYGASNRYTGVPDRFTGSGSATDFTLTISSVQAEDLADYHCGQGYSYPYTFGGGTKLEIKRTVAAPSVFIFPPSDEQLKSGTASVVCLLNNFYPREAKVQWKVDNALQSGNSQESVTEQDSKDSTYSLSSTLTLSKADYEKHKVYACEVTHQGLSSPVTKSFNRGECGGGGSGGGGSGGGGSAIVMTQTPSSKSVPVGDTVTINCQASESVDRNNRLAWFQQKPGQPPKLLIYTTSTLASGVPSRFKGSGSGTHFTLTISDVVPDDAATYYCAGYRGAHTDGDAFGCGTEVVVKGGGGSGGGGSGGGGSGGGGSQSLEESGGDLVKPGASLTLTCTASGFSFSRSSYMCWVRQAPGKCLEWIGCLSVGDGHTYYASWAKGRFTISKTSSTSVTLQMTRLTAADTATYFCARAPSYSGDGGHGYDLWGPGTLVTVSS

SEQ ID NO: 162 - protein, 446 aa, synthetic construct; identical to SEQ ID NO: 160

SEQ ID NO: 163 - protein, 214 aa, synthetic construct
NIVMTQSPKSMSMSVGERVTLTCKASENVVTYVSWYQQKPEQSPKLLIYGASNRYTGVPDRFTGSGSATDFTLTISSVQAEDLADYHCGQGYSYPYTFGGGTKLEIKRTVAAPSVFIFPPSDEQLKSGTASVVCLLNNFYPREAKVQWKVDNALQSGNSQESVTEQDSKDSTYSLSSTLTLSKADYEKHKVYACEVTHQGLSSPVTKSFNRGEC

SEQ ID NO: 164 - protein, 5 aa, synthetic construct
GYTMN

SEQ ID NO: 165 - protein, 7 aa, synthetic construct
GYSFTGY

SEQ ID NO: 166 - protein, 17 aa, synthetic construct
LINPYNSDTNYAQKLQG

SEQ ID NO: 167 - protein, 6 aa, synthetic construct
NPYNSD

SEQ ID NO: 168 - protein, 9 aa, synthetic construct
VALRVALDY

SEQ ID NO: 169 - protein, 11 aa, synthetic construct
KASQNVATHVG

SEQ ID NO: 170 - protein, 7 aa, synthetic construct
SASYRYS

SEQ ID NO: 171 - protein, 9 aa, synthetic construct
QQYNRYPYT

SEQ ID NO: 172 - protein, 118 aa, synthetic construct
QVQLVQSGAEVKKPGASVKVSCKASGYSFTGYTMNWVRQAPGQGLEWMGLINPYNSDTNYAQKLQGRVTMTTDTSTSTAYMELRSLRSDDTAVYYCARVALRVALDYWGQGTLVTVSS

SEQ ID NO: 173 - protein, 107 aa, synthetic construct
DIQMTQSPSSLSASVGDRVTITCKASQNVATHVGWYQQKPGKAPKRLIYSASYRYSGVPSRFSGSGSGTEFTLTISNLQPEDFATYYCQQYNRYPYTFGQGTKLEIK

SEQ ID NO: 174 - protein, 448 aa, synthetic construct
QVQLVQSGAEVKKPGASVKVSCKASGYSFTGYTMNWVRQAPGQGLEWMGLINPYNSDTNYAQKLQGRVTMTTDTSTSTAYMELRSLRSDDTAVYYCARVALRVALDYWGQGTLVTVSSASTKGPSVFPLAPSSKSTSGGTAALGCLVKDYFPEPVTVSWNSGALTSGVHTFPAVLQSSGLYSLSSVVTVPSSSLGTQTYICNVNHKPSNTKVDKKVEPKSCDKTHTCPPCPAPELLAGPSVFLFPPKPKDTLMISRTPEVTCVVVDVSHEDPEVKFNWYVDGVEVHNAKTKPREEQYNSTYRVVSVLTVLHQDWLNGKEYKCKVSNKALPLPEEKTISKAKGQPREPQVYTLPPSRDELTKNQVSLTCLVKGFYPSDIAVEWESNGQPENNYKTTPPVLDSDGSFFLYSKLTVDKSRWQQGNVFSCSVMHEALHNHYTQKSLSLSPGK

SEQ ID NO: 175 - protein, 485 aa, synthetic construct
DIQMTQSPSSLSASVGDRVTITCKASQNVATHVGWYQQKPGKAPKRLIYSASYRYSGVPSRFSGSGSGTEFTLTISNLQPEDFATYYCQQYNRYPYTFGQGTKLEIKRTVAAPSVFIFPPSDEQLKSGTASVVCLLNNFYPREAKVQWKVDNALQSGNSQESVTEQDSKDSTYSLSSTLTLSKADYEKHKVYACEVTHQGLSSPVTKSFNRGECGGGGSGGGGSGGGGSDIQMTQSPSSLSASVGDRVTITCQASESVDRNNRLAWFQQKPGKPPKLLIYTTSTLASGVPSRFSGSGSGTDFTLTISSLQPEDVATYYCAGYRGAHTDGDAFGCGTKVEIKGGGGSGGGGSGGGGSGGGGSEQQLVESGGGLVKPGGSLRLSCAASGFSFSRSSYMCWVRQAPGKCLEWIGCLSVGDGHTYYASWAKGRFTISKDSAKNSVYLQMNSLRAEDTAVYFCARAPSYSGDGGHGYDLWGPGTLVTVSS

SEQ ID NO: 176 - protein, 7 aa, synthetic construct
SGSYFWG

SEQ ID NO: 177 - protein, 9 aa, synthetic construct
GGSISSGSY

SEQ ID NO: 178 - protein, 16 aa, synthetic construct
SIYYSGITYYNPSLKS

SEQ ID NO: 179 - protein, 5 aa, synthetic construct
YYSGI

SEQ ID NO: 180 - protein, 11 aa, synthetic construct
HDGAVAGLFDY

SEQ ID NO: 181 - protein, 11 aa, synthetic construct
GGNNIGSKSVH

SEQ ID NO: 182 - protein, 7 aa, synthetic construct
DDSDRPS

SEQ ID NO: 183 - protein, 11 aa, synthetic construct
QVWDSSSDHVV

SEQ ID NO: 184 - protein, 121 aa, synthetic construct
QLQLQESGPGLVKPSETLSLTCTVSGGSISSGSYFWGWIRQPPGKGLEWIGSIYYSGITYYNPSLKSRVTISVDTSKNQFSLKLSSVTAADTAVYYCARHDGAVAGLFDYWGQGTLVTVSS

SEQ ID NO: 185 - protein, 111 aa, synthetic construct
SYVLTQPPSVSVAPGQTARITCGGNNIGSKSVHWYQQPPGQAPVVVVYDDSDRPSGIPERFSGSNSGNTATLTISRVEAGDEAVYYCQVWDSSSDHVVFGGGTKLTVLGQP

SEQ ID NO: 186 - protein, 451 aa, synthetic construct
QLQLQESGPGLVKPSETLSLTCTVSGGSISSGSYFWGWIRQPPGKGLEWIGSIYYSGITYYNPSLKSRVTISVDTSKNQFSLKLSSVTAADTAVYYCARHDGAVAGLFDYWGQGTLVTVSSASTKGPSVFPLAPSSKSTSGGTAALGCLVKDYFPEPVTVSWNSGALTSGVHTFPAVLQSSGLYSLSSVVTVPSSSLGTQTYICNVNHKPSNTKVDKKVEPKSCDKTHTCPPCPAPELLAGPSVFLFPPKPKDTLMISRTPEVTCVVVDVSHEDPEVKFNWYVDGVEVHNAKTKPREEQYNSTYRVVSVLTVLHQDWLNGKEYKCKVSNKALPLPEEKTISKAKGQPREPQVYTLPPSRDELTKNQVSLTCLVKGFYPSDIAVEWESNGQPENNYKTTPPVLDSDGSFFLYSKLTVDKSRWQQGNVFSCSVMHEALHNHYTQKSLSLSPGK

SEQ ID NO: 187 - protein, 485 aa, synthetic construct
SYVLTQPPSVSVAPGQTARITCGGNNIGSKSVHWYQQPPGQAPVVVVYDDSDRPSGIPERFSGSNSGNTATLTISRVEAGDEAVYYCQVWDSSSDHVVFGGGTKLTVLGQPKAAPSVTLFPPSSEELQANKATLVCLISDFYPGAVTVAWKGDSSPVKAGVETTTPSKQSNNKYAASSYLSLTPEQWKSHRSYSCQVTHEGSTVEKTVAPTECSGGGGSGGGGSGGGGSDIQMTQSPSSLSASVGDRVTITCQASESVDRNNRLAWFQQKPGKPPKLLIYTTSTLASGVPSRFSGSGSGTDFTLTISSLQPEDVATYYCAGYRGAHTDGDAFGCGTKVEIKGGGGSGGGGSGGGGSGGGGSEQQLVESGGGLVKPGGSLRLSCAASGFSFSRSSYMCWVRQAPGKCLEWIGCLSVGDGHTYYASWAKGRFTISKDSAKNSVYLQMNSLRAEDTAVYFCARAPSYSGDGGHGYDLWGPGTLVTVSS

SEQ ID NO: 188 - protein, 5 aa, synthetic construct
SFAMS

SEQ ID NO: 189 - protein, 7 aa, synthetic construct
GFTFNSF

SEQ ID NO: 190 - protein, 17 aa, synthetic construct
AISGSGGGTYYADSVKG

SEQ ID NO: 191 - protein, 6 aa, synthetic construct
SGSGGG

SEQ ID NO: 192 - protein, 13 aa, synthetic construct
DKILWFGEPVFDY

SEQ ID NO: 193 - protein, 11 aa, synthetic construct
RASQSVSSYLA

SEQ ID NO: 194 - protein, 7 aa, synthetic construct
DASNRAT

SEQ ID NO: 195 - protein, 9 aa, synthetic construct
QQRSNWPPT

SEQ ID NO: 196 - protein, 122 aa, synthetic construct [sequence omitted]

SEQ ID NO: 197 - protein, 107 aa, synthetic construct [sequence omitted]

SEQ ID NO: 198 - protein, 452 aa, synthetic construct
EVQLLESGGGLVQPGGSLRLSCAVSGFTFNSFAMSWVRQAPGKGLEWVSAISGSGGGTYYADSVKGRFTISRDNSKNTLYLQMNSLRAEDTAVYFCAKDKILWFGEPVFDYWGQGTLVTVSSASTKGPSVFPLAPSSKSTSGGTAALGCLVKDYFPEPVTVSWNSGALTSGVHTFPAVLQSSGLYSLSSVVTVPSSSLGTQTYICNVNHKPSNTKVDKKVEPKSCDKTHTCPPCPAPELLAGPSVFLFPPKPKDTLMISRTPEVTCVVVDVSHEDPEVKFNWYVDGVEVHNAKTKPREEQYNSTYRVVSVLTVLHQDWLNGKEYKCKVSNKALPLPEEKTISKAKGQPREPQVYTLPPSRDELTKNQVSLTCLVKGFYPSDIAVEWESNGQPENNYKTTPPVLDSDGSFFLYSKLTVDKSRWQQGNVFSCSVMHEALHNHYTQKSLSLSPGK

SEQ ID NO: 199 - protein, 485 aa, synthetic construct
EIVLTQSPATLSLSPGERATLSCRASQSVSSYLAWYQQKPGQAPRLLIYDASNRATGIPARFSGSGSGTDFTLTISSLEPEDFAVYYCQQRSNWPPTFGQGTKVEIKRTVAAPSVFIFPPSDEQLKSGTASVVCLLNNFYPREAKVQWKVDNALQSGNSQESVTEQDSKDSTYSLSSTLTLSKADYEKHKVYACEVTHQGLSSPVTKSFNRGECGGGGSGGGGSGGGGSDIQMTQSPSSLSASVGDRVTITCQASESVDRNNRLAWFQQKPGKPPKLLIYTTSTLASGVPSRFSGSGSGTDFTLTISSLQPEDVATYYCAGYRGAHTDGDAFGCGTKVEIKGGGGSGGGGSGGGGSGGGGSEQQLVESGGGLVKPGGSLRLSCAASGFSFSRSSYMCWVRQAPGKCLEWIGCLSVGDGHTYYASWAKGRFTISKDSAKNSVYLQMNSLRAEDTAVYFCARAPSYSGDGGHGYDLWGPGTLVTVSS

SEQ ID NO: 200 - protein, 6 aa, synthetic construct
IDYWIS

SEQ ID NO: 201 - protein, 8 aa, synthetic construct
GFTINIDY

SEQ ID NO: 202 - protein, 17 aa, synthetic construct
IIDPGDGTTYFAIWVSG

SEQ ID NO: 203 - protein, 6 aa, synthetic construct
DPGDGT

SEQ ID NO: 204 - protein, 11 aa, synthetic construct
EFSASAYQYDL

SEQ ID NO: 205 - protein, 11 aa, synthetic construct
RASEDIENYLA

SEQ ID NO: 206 - protein, 7 aa, synthetic construct
RASTLSS

SEQ ID NO: 207 - protein, 12 aa, synthetic construct
QQGYRNSNVDNP

SEQ ID NO: 208 - protein, 121 aa, synthetic construct
EQQLVETGGGLIQPGGSLRLSCAASGFTINIDYWISWVRQAPGKGLEWIGIIDPGDGTTYFAIWVSGRFTISFDNSKNTVYLQMNSLRAEDTAVYFCVREFSASAYQYDLWGPGTLVTVSS

SEQ ID NO: 209 - protein, 110 aa, synthetic construct
ELVMTQSPATLSVSPGERATLSCRASEDIENYLAWYQQKPGQPPRLLIYRASTLSSGVPARFSGSGSGTEFTLTISSLQSEDFAVYYCQQGYRNSNVDNPFGGGTKVEIK

SEQ ID NO: 210 - protein, 451 aa, synthetic construct
EQQLVETGGGLIQPGGSLRLSCAASGFTINIDYWISWVRQAPGKGLEWIGIIDPGDGTTYFAIWVSGRFTISFDNSKNTVYLQMNSLRAEDTAVYFCVREFSASAYQYDLWGPGTLVTVSSASTKGPSVFPLAPSSKSTSGGTAALGCLVKDYFPEPVTVSWNSGALTSGVHTFPAVLQSSGLYSLSSVVTVPSSSLGTQTYICNVNHKPSNTKVDKKVEPKSCDKTHTCPPCPAPEAAGGPSVFLFPPKPKDTLMISRTPEVTCVVVDVSHEDPEVKFNWYVDGVEVHNAKTKPREEQYNSTYRVVSVLTVLHQDWLNGKEYKCKVSNKALGAPIEKTISKAKGQPREPQVCTLPPSRDELTKNQVSLSCAVKGFYPSDIAVEWESNGQPENNYKTTPPVLDSDGSFFLVSKLTVDKSRWQQGNVFSCSVMHEALHNRFTQKSLSLSPGK

SEQ ID NO: 211 - protein, 454 aa, synthetic construct
EQQLVESGGGLVKPGGSLRLSCAASGFSFSRSSYMCWVRQAPGKGLEWIGCLSVGDGHTYYASWAKGRFTISKDSAKNSVYLQMNSLRAEDTAVYFCARAPSYSGDGGHGYDLWGPGTLVTVSSASTKGPSVFPLAPSSKSTSGGTAALGCLVKDYFPEPVTVSWNSGALTSGVHTFPAVLQSSGLYSLSSVVTVPSSSLGTQTYICNVNHKPSNTKVDKKVEPKSCDKTHTCPPCPAPEAAGGPSVFLFPPKPKDTLMISRTPEVTCVVVDVSHEDPEVKFNWYVDGVEVHNAKTKPREEQYNSTYRVVSVLTVLHQDWLNGKEYKCKVSNKALGAPIEKTISKAKGQPREPQVYTLPPCRDELTKNQVSLWCLVKGFYPSDIAVEWESNGQPENNYKTTPPVLDSDGSFFLYSKLTVDKSRWQQGNVFSCSVMHEALHNHYTQKSLSLSPGK

SEQ ID NO: 212 - protein, 217 aa, synthetic construct
ELVMTQSPATLSVSPGERATLSCRASEDIENYLAWYQQKPGQPPRLLIYRASTLSSGVPARFSGSGSGTEFTLTISSLQSEDFAVYYCQQGYRNSNVDNPFGGGTKVEIKRTVAAPSVFIFPPSDEQLKSGTASVVCLLNNFYPREAKVQWKVDNALQSGNSQESVTEQDSKDSTYSLSSTLTLSKADYEKHKVYACEVTHQGLSSPVTKSFNRGEC

SEQ ID NO: 213 - protein, 219 aa, synthetic construct
DIQMTQSPSSLSASVGDRVTITCQASESVDRNNRLAWFQQKPGKPPKLLIYTTSTLASGVPSRFSGSGSGTDFTLTISSLQPEDVATYYCAGYRGAHTDGDAFGGGTKVEIKRTVAAPSVFIFPPSDEQLKSGTASVVCLLNNFYPREAKVQWKVDNALQSGNSQESVTEQDSKDSTYSLSSTLTLSKADYEKHKVYACEVTHQGLSSPVTKSFNRGEC

SEQ ID NO: 214 - protein, 451 aa, synthetic construct; identical to SEQ ID NO: 210

SEQ ID NO: 215 - protein, 483 aa, synthetic construct
DIQMTQSPSSLSASVGDRVTITCQASESVDRNNRLAWFQQKPGKPPKLLIYTTSTLASGVPSRFSGSGSGTDFTLTISSLQPEDVATYYCAGYRGAHTDGDAFGGGTKVEIKGGGGSGGGGSGGGGSGGGGSEQQLVESGGGLVKPGGSLRLSCAASGFSFSRSSYMCWVRQAPGKGLEWIGCLSVGDGHTYYASWAKGRFTISKDSAKNSVYLQMNSLRAEDTAVYFCARAPSYSGDGGHGYDLWGPGTLVTVSSDKTHTCPPCPAPEAAGGPSVFLFPPKPKDTLMISRTPEVTCVVVDVSHEDPEVKFNWYVDGVEVHNAKTKPREEQYNSTYRVVSVLTVLHQDWLNGKEYKCKVSNKALGAPIEKTISKAKGQPREPQVYTLPPCRDELTKNQVSLWCLVKGFYPSDIAVEWESNGQPENNYKTTPPVLDSDGSFFLYSKLTVDKSRWQQGNVFSCSVMHEALHNHYTQKSLSLSPGK

SEQ ID NO: 216 - protein, 217 aa, synthetic construct; identical to SEQ ID NO: 212

SEQ ID NO: 217 - protein, 691 aa, synthetic construct
EQQLVETGGGLIQPGGSLRLSCAASGFTINIDYWISWVRQAPGKGLEWIGIIDPGDGTTYFAIWVSGRFTISFDNSKNTVYLQMNSLRAEDTAVYFCVREFSASAYQYDLWGPGTLVTVSSASTKGPSVFPLAPSSKSTSGGTAALGCLVKDYFPEPVTVSWNSGALTSGVHTFPAVLQSSGLYSLSSVVTVPSSSLGTQTYICNVNHKPSNTKVDKKVEPKSCDGGGGSGGGGSGGGGSEQQLVETGGGLIQPGGSLRLSCAASGFTINIDYWISWVRQAPGKGLEWIGIIDPGDGTTYFAIWVSGRFTISFDNSKNTVYLQMNSLRAEDTAVYFCVREFSASAYQYDLWGPGTLVTVSSASTKGPSVFPLAPSSKSTSGGTAALGCLVKDYFPEPVTVSWNSGALTSGVHTFPAVLQSSGLYSLSSVVTVPSSSLGTQTYICNVNHKPSNTKVDKKVEPKSCDKTHTCPPCPAPEAAGGPSVFLFPPKPKDTLMISRTPEVTCVVVDVSHEDPEVKFNWYVDGVEVHNAKTKPREEQYNSTYRVVSVLTVLHQDWLNGKEYKCKVSNKALGAPIEKTISKAKGQPREPQVCTLPPSRDELTKNQVSLSCAVKGFYPSDIAVEWESNGQPENNYKTTPPVLDSDGSFFLVSKLTVDKSRWQQGNVFSCSVMHEALHNRFTQKSLSLSPGK

SEQ ID NO: 218 - protein, 483 aa, synthetic construct; identical to SEQ ID NO: 215

SEQ ID NO: 219 - protein, 217 aa, synthetic construct; identical to SEQ ID NO: 212

SEQ ID NO: 220 - protein, 451 aa, synthetic construct; identical to SEQ ID NO: 210

SEQ ID NO: 221 - protein, 722 aa, synthetic construct
EQQLVETGGGLIQPGGSLRLSCAASGFTINIDYWISWVRQAPGKGLEWIGIIDPGDGTTYFAIWVSGRFTISFDNSKNTVYLQMNSLRAEDTAVYFCVREFSASAYQYDLWGPGTLVTVSSASTKGPSVFPLAPSSKSTSGGTAALGCLVKDYFPEPVTVSWNSGALTSGVHTFPAVLQSSGLYSLSSVVTVPSSSLGTQTYICNVNHKPSNTKVDKKVEPKSCDKTHTCPPCPAPEAAGGPSVFLFPPKPKDTLMISRTPEVTCVVVDVSHEDPEVKFNWYVDGVEVHNAKTKPREEQYNSTYRVVSVLTVLHQDWLNGKEYKCKVSNKALGAPIEKTISKAKGQPREPQVYTLPPCRDELTKNQVSLWCLVKGFYPSDIAVEWESNGQPENNYKTTPPVLDSDGSFFLYSKLTVDKSRWQQGNVFSCSVMHEALHNHYTQKSLSLSPGKGGGGSGGGGSGGGGSDIQMTQSPSSLSASVGDRVTITCQASESVDRNNRLAWFQQKPGKPPKLLIYTTSTLASGVPSRFSGSGSGTDFTLTISSLQPEDVATYYCAGYRGAHTDGDAFGGGTKVEIKGGGGSGGGGSGGGGSGGGGSEQQLVESGGGLVKPGGSLRLSCAASGFSFSRSSYMCWVRQAPGKGLEWIGCLSVGDGHTYYASWAKGRFTISKDSAKNSVYLQMNSLRAEDTAVYFCARAPSYSGDGGHGYDLWGPGTLVTVSS

SEQ ID NO: 222 - protein, 217 aa, synthetic construct; identical to SEQ ID NO: 212

SEQ ID NO: 223 - protein, 451 aa, synthetic construct
EQQLVETGGGLIQPGGSLRLSCAASGFTINIDYWISWVRQAPGKGLEWIGIIDPGDGTTYFAIWVSGRFTISFDNSKNTVYLQMNSLRAEDTAVYFCVREFSASAYQYDLWGPGTLVTVSSASTKGPSVFPLAPSSKSTSGGTAALGCLVKDYFPEPVTVSWNSGALTSGVHTFPAVLQSSGLYSLSSVVTVPSSSLGTQTYICNVNHKPSNTKVDKKVEPKSCDKTHTCPPCPAPEAAGGPSVFLFPPKPKDTLMISRTPEVTCVVVDVSHEDPEVKFNWYVDGVEVHNAKTKPREEQYNSTYRVVSVLTVLHQDWLNGKEYKCKVSNKALGAPIEKTISKAKGQPREPQVYTLPPSRDELTKNQVSLTCLVKGFYPSDIAVEWESNGQPENNYKTTPPVLDSDGSFFLYSKLTVDKSRWQQGNVFSCSVMHEALHNHYTQKSLSLSPGK

SEQ ID NO: 224 - protein, 488 aa, synthetic construct
ELVMTQSPATLSVSPGERATLSCRASEDIENYLAWYQQKPGQPPRLLIYRASTLSSGVPARFSGSGSGTEFTLTISSLQSEDFAVYYCQQGYRNSNVDNPFGGGTKVEIKRTVAAPSVFIFPPSDEQLKSGTASVVCLLNNFYPREAKVQWKVDNALQSGNSQESVTEQDSKDSTYSLSSTLTLSKADYEKHKVYACEVTHQGLSSPVTKSFNRGECGGGGSGGGGSGGGGSDIQMTQSPSSLSASVGDRVTITCQASESVDRNNRLAWFQQKPGKPPKLLIYTTSTLASGVPSRFSGSGSGTDFTLTISSLQPEDVATYYCAGYRGAHTDGDAFGGGTKVEIKGGGGSGGGGSGGGGSGGGGSEQQLVESGGGLVKPGGSLRLSCAASGFSFSRSSYMCWVRQAPGKGLEWIGCLSVGDGHTYYASWAKGRFTISKDSAKNSVYLQMNSLRAEDTAVYFCARAPSYSGDGGHGYDLWGPGTLVTVSS

SEQ ID NO: 225 - protein, 722 aa, synthetic construct
EQQLVETGGGLIQPGGSLRLSCAASGFTINIDYWISWVRQAPGKGLEWIGIIDPGDGTTYFAIWVSGRFTISFDNSKNTVYLQMNSLRAEDTAVYFCVREFSASAYQYDLWGPGTLVTVSSASTKGPSVFPLAPSSKSTSGGTAALGCLVKDYFPEPVTVSWNSGALTSGVHTFPAVLQSSGLYSLSSVVTVPSSSLGTQTYICNVNHKPSNTKVDKKVEPKSCDKTHTCPPCPAPEAAGGPSVFLFPPKPKDTLMISRTPEVTCVVVDVSHEDPEVKFNWYVDGVEVHNAKTKPREEQYNSTYRVVSVLTVLHQDWLNGKEYKCKVSNKALGAPIEKTISKAKGQPREPQVYTLPPSRDELTKNQVSLTCLVKGFYPSDIAVEWESNGQPENNYKTTPPVLDSDGSFFLYSKLTVDKSRWQQGNVFSCSVMHEALHNHYTQKSLSLSPGKGGGGSGGGGSGGGGSDIQMTQSPSSLSASVGDRVTITCQASESVDRNNRLAWFQQKPGKPPKLLIYTTSTLASGVPSRFSGSGSGTDFTLTISSLQPEDVATYYCAGYRGAHTDGDAFGGGTKVEIKGGGGSGGGGSGGGGSGGGGSEQQLVESGGGLVKPGGSLRLSCAASGFSFSRSSYMCWVRQAPGKGLEWIGCLSVGDGHTYYASWAKGRFTISKDSAKNSVYLQMNSLRAEDTAVYFCARAPSYSGDGGHGYDLWGPGTLVTVSS

SEQ ID NO: 226 - protein, 217 aa, synthetic construct; identical to SEQ ID NO: 212

SEQ ID NO: 227 - protein, 451 aa, synthetic construct
EQQLVETGGGLIQPGGSLRLSCAASGFTINIDYWISWVRQAPGKGLEWIGIIDPGDGTTYFAIWVSGRFTISFDNSKNTVYLQMNSLRAEDTAVYFCVREFSASAYQYDLWGPGTLVTVSSASTKGPSVFPLAPSSKSTSGGTAALGCLVKDYFPEPVTVSWNSGALTSGVHTFPAVLQSSGLYSLSSVVTVPSSSLGTQTYICNVNHKPSNTKVDKKVEPKSCDKTHTCPPCPAPELLAGPSVFLFPPKPKDTLMISRTPEVTCVVVDVSHEDPEVKFNWYVDGVEVHNAKTKPREEQYNSTYRVVSVLTVLHQDWLNGKEYKCKVSNKALPLPEEKTISKAKGQPREPQVYTLPPSRDELTKNQVSLSCAVKGFYPSDIAVEWESNGQPENNYKTTPPVLDSDGSFFLVSKLTVDKSRWQQGNVFSCSVMHEALHNHYTQKSLSLSPGK

SEQ ID NO: 228 - protein, 454 aa, synthetic construct
EQQLVESGGGLVKPGGSLRLSCAASGFSFSRSSYMCWVRQAPGKGLEWIGCLSVGDGHTYYASWAKGRFTISKDSAKNSVYLQMNSLRAEDTAVYFCARAPSYSGDGGHGYDLWGPGTLVTVSSASTKGPSVFPLAPSSKSTSGGTAALGCLVKDYFPEPVTVSWNSGALTSGVHTFPAVLQSSGLYSLSSVVTVPSSSLGTQTYICNVNHKPSNTKVDKKVEPKSCDKTHTCPPCPAPELLAGPSVFLFPPKPKDTLMISRTPEVTCVVVDVSHEDPEVKFNWYVDGVEVHNAKTKPREEQYNSTYRVVSVLTVLHQDWLNGKEYKCKVSNKALPLPEEKTISKAKGQPREPQVYTLPPSRDELTKNQVSLWCLVKGFYPSDIAVEWESNGQPENNYKTTPPVLDSDGSFFLYSKLTVDKSRWQQGNVFSCSVMHEALHNHYTQKSLSLSPGK

SEQ ID NO: 229 - protein, 217 aa, synthetic construct; identical to SEQ ID NO: 212

SEQ ID NO: 230 - protein, 219 aa, synthetic construct; identical to SEQ ID NO: 213

SEQ ID NO: 231 - protein, 451 aa, synthetic construct; identical to SEQ ID NO: 227

SEQ ID NO: 232 - protein, 483 aa, synthetic construct
DIQMTQSPSSLSASVGDRVTITCQASESVDRNNRLAWFQQKPGKPPKLLIYTTSTLASGVPSRFSGSGSGTDFTLTISSLQPEDVATYYCAGYRGAHTDGDAFGGGTKVEIKGGGGSGGGGSGGGGSGGGGSEQQLVESGGGLVKPGGSLRLSCAASGFSFSRSSYMCWVRQAPGKGLEWIGCLSVGDGHTYYASWAKGRFTISKDSAKNSVYLQMNSLRAEDTAVYFCARAPSYSGDGGHGYDLWGPGTLVTVSSDKTHTCPPCPAPELLAGPSVFLFPPKPKDTLMISRTPEVTCVVVDVSHEDPEVKFNWYVDGVEVHNAKTKPREEQYNSTYRVVSVLTVLHQDWLNGKEYKCKVSNKALPLPEEKTISKAKGQPREPQVYTLPPSRDELTKNQVSLWCLVKGFYPSDIAVEWESNGQPENNYKTTPPVLDSDGSFFLYSKLTVDKSRWQQGNVFSCSVMHEALHNHYTQKSLSLSPGK

SEQ ID NO: 233 - protein, 217 aa, synthetic construct; identical to SEQ ID NO: 212

SEQ ID NO: 234 - protein, 691 aa, synthetic construct
EQQLVETGGGLIQPGGSLRLSCAASGFTINIDYWISWVRQAPGKGLEWIGIIDPGDGTTYFAIWVSGRFTISFDNSKNTVYLQMNSLRAEDTAVYFCVREFSASAYQYDLWGPGTLVTVSSASTKGPSVFPLAPSSKSTSGGTAALGCLVKDYFPEPVTVSWNSGALTSGVHTFPAVLQSSGLYSLSSVVTVPSSSLGTQTYICNVNHKPSNTKVDKKVEPKSCDGGGGSGGGGSGGGGSEQQLVETGGGLIQPGGSLRLSCAASGFTINIDYWISWVRQAPGKGLEWIGIIDPGDGTTYFAIWVSGRFTISFDNSKNTVYLQMNSLRAEDTAVYFCVREFSASAYQYDLWGPGTLVTVSSASTKGPSVFPLAPSSKSTSGGTAALGCLVKDYFPEPVTVSWNSGALTSGVHTFPAVLQSSGLYSLSSVVTVPSSSLGTQTYICNVNHKPSNTKVDKKVEPKSCDKTHTCPPCPAPELLAGPSVFLFPPKPKDTLMISRTPEVTCVVVDVSHEDPEVKFNWYVDGVEVHNAKTKPREEQYNSTYRVVSVLTVLHQDWLNGKEYKCKVSNKALPLPEEKTISKAKGQPREPQVYTLPPSRDELTKNQVSLSCAVKGFYPSDIAVEWESNGQPENNYKTTPPVLDSDGSFFLVSKLTVDKSRWQQGNVFSCSVMHEALHNHYTQKSLSLSPGK

SEQ ID NO: 235 - protein, 483 aa, synthetic construct; identical to SEQ ID NO: 232

SEQ ID NO: 236 - protein, 217 aa, synthetic construct; identical to SEQ ID NO: 212

SEQ ID NO: 237 - protein, 451 aa, synthetic construct; identical to SEQ ID NO: 227

SEQ ID NO: 238 - protein, 722 aa, synthetic construct
EQQLVETGGGLIQPGGSLRLSCAASGFTINIDYWISWVRQAPGKGLEWIGIIDPGDGTTYFAIWVSGRFTISFDNSKNTVYLQMNSLRAEDTAVYFCVREFSASAYQYDLWGPGTLVTVSSASTKGPSVFPLAPSSKSTSGGTAALGCLVKDYFPEPVTVSWNSGALTSGVHTFPAVLQSSGLYSLSSVVTVPSSSLGTQTYICNVNHKPSNTKVDKKVEPKSCDKTHTCPPCPAPELLAGPSVFLFPPKPKDTLMISRTPEVTCVVVDVSHEDPEVKFNWYVDGVEVHNAKTKPREEQYNSTYRVVSVLTVLHQDWLNGKEYKCKVSNKALPLPEEKTISKAKGQPREPQVYTLPPSRDELTKNQVSLWCLVKGFYPSDIAVEWESNGQPENNYKTTPPVLDSDGSFFLYSKLTVDKSRWQQGNVFSCSVMHEALHNHYTQKSLSLSPGKGGGGSGGGGSGGGGSDIQMTQSPSSLSASVGDRVTITCQASESVDRNNRLAWFQQKPGKPPKLLIYTTSTLASGVPSRFSGSGSGTDFTLTISSLQPEDVATYYCAGYRGAHTDGDAFGGGTKVEIKGGGGSGGGGSGGGGSGGGGSEQQLVESGGGLVKPGGSLRLSCAASGFSFSRSSYMCWVRQAPGKGLEWIGCLSVGDGHTYYASWAKGRFTISKDSAKNSVYLQMNSLRAEDTAVYFCARAPSYSGDGGHGYDLWGPGTLVTVSS

SEQ ID NO: 239 - protein, 217 aa, synthetic construct; identical to SEQ ID NO: 212

SEQ ID NO: 240 - protein, 451 aa, synthetic construct
EQQLVETGGGLIQPGGSLRLSCAASGFTINIDYWISWVRQAPGKGLEWIGIIDPGDGTTYFAIWVSGRFTISFDNSKNTVYLQMNSLRAEDTAVYFCVREFSASAYQYDLWGPGTLVTVSSASTKGPSVFPLAPSSKSTSGGTAALGCLVKDYFPEPVTVSWNSGALTSGVHTFPAVLQSSGLYSLSSVVTVPSSSLGTQTYICNVNHKPSNTKVDKKVEPKSCDKTHTCPPCPAPELLAGPSVFLFPPKPKDTLMISRTPEVTCVVVDVSHEDPEVKFNWYVDGVEVHNAKTKPREEQYNSTYRVVSVLTVLHQDWLNGKEYKCKVSNKALPLPEEKTISKAKGQPREPQVYTLPPSRDELTKNQVSLTCLVKGFYPSDIAVEWESNGQPENNYKTTPPVLDSDGSFFLYSKLTVDKSRWQQGNVFSCSVMHEALHNHYTQKSLSLSPGK

SEQ ID NO: 241 - protein, 488 aa, synthetic construct
ELVMTQSPATLSVSPGERATLSCRASEDIENYLAWYQQKPGQPPRLLIYRASTLSSGVPARFSGSGSGTEFTLTISSLQSEDFAVYYCQQGYRNSNVDNPFGGGTKVEIKRTVAAPSVFIFPPSDEQLKSGTASVVCLLNNFYPREAKVQWKVDNALQSGNSQESVTEQDSKDSTYSLSSTLTLSKADYEKHKVYACEVTHQGLSSPVTKSFNRGECGGGGSGGGGSGGGGSDIQMTQSPSSLSASVGDRVTITCQASESVDRNNRLAWFQQKPGKPPKLLIYTTSTLASGVPSRFSGSGSGTDFTLTISSLQPEDVATYYCAGYRGAHTDGDAFGCGTKVEIKGGGGSGGGGSGGGGSGGGGSEQQLVESGGGLVKPGGSLRLSCAASGFSFSRSSYMCWVRQAPGKCLEWIGCLSVGDGHTYYASWAKGRFTISKDSAKNSVYLQMNSLRAEDTAVYFCARAPSYSGDGGHGYDLWGPGTLVTVSS

SEQ ID NO: 242 - protein, 721 aa, synthetic construct
EQQLVETGGGLIQPGGSLRLSCAASGFTINIDYWISWVRQAPGKGLEWIGIIDPGDGTTYFAIWVSGRFTISFDNSKNTVYLQMNSLRAEDTAVYFCVREFSASAYQYDLWGPGTLVTVSSASTKGPSVFPLAPSSKSTSGGTAALGCLVKDYFPEPVTVSWNSGALTSGVHTFPAVLQSSGLYSLSSVVTVPSSSLGTQTYICNVNHKPSNTKVDKKVEPKSCDKTHTCPPCPAPELLAGPSVFLFPPKPKDTLMISRTPEVTCVVVDVSHEDPEVKFNWYVDGVEVHNAKTKPREEQYNSTYRVVSVLTVLHQDWLNGKEYKCKVSNKALPLPEEKTISKAKGQPREPQVYTLPPSRDELTKNQVSLTCLVKGFYPSDIAVEWESNGQPENNYKTTPPVLDSDGSFFLYSKLTVDKSRWQQGNVFSCSVMHEALHNHYTQKSLSLSPGGGGGSGGGGSGGGGSDIQMTQSPSSLSASVGDRVTITCQASESVDRNNRLAWFQQKPGKPPKLLIYTTSTLASGVPSRFSGSGSGTDFTLTISSLQPEDVATYYCAGYRGAHTDGDAFGCGTKVEIKGGGGSGGGGSGGGGSGGGGSEQQLVESGGGLVKPGGSLRLSCAASGFSFSRSSYMCWVRQAPGKCLEWIGCLSVGDGHTYYASWAKGRFTISKDSAKNSVYLQMNSLRAEDTAVYFCARAPSYSGDGGHGYDLWGPGTLVTVSS

SEQ ID NO: 243 - protein, 217 aa, synthetic construct; identical to SEQ ID NO: 212

SEQ ID NO: 244 - protein, 722 aa, synthetic construct
QSLEESGGDLVKPGASLTLTCTASGFSFSGMYWICWVRQAPGKGLEWIACIYTGSSTTGYASWAKGRFTISKTSSTTVTLQMTSLTAADTATHFCASPYGDSSHYRGLNLWGPGTLVTVSSASTKGPSVFPLAPSSKSTSGGTAALGCLVKDYFPEPVTVSWNSGALTSGVHTFPAVLQSSGLYSLSSVVTVPSSSLGTQTYICNVNHKPSNTKVDKKVEPKSCDKTHTCPPCPAPEAAGGPSVFLFPPKPKDTLMISRTPEVTCVVVDVSHEDPEVKFNWYVDGVEVHNAKTKPREEQYNSTYRVVSVLTVLHQDWLNGKEYKCKVSNKALGAPIEKTISKAKGQPREPQVYTLPPSRDELTKNQVSLTCLVKGFYPSDIAVEWESNGQPENNYKTTPPVLDSDGSFFLYSKLTVDKSRWQQGNVFSCSVMHEALHNHYTQKSLSLSPGKGGGGSGGGGSGGGGSDIQMTQSPSSLSASVGDRVTITCQASESVDRNNRLAWFQQKPGKPPKLLIYTTSTLASGVPSRFSGSGSGTDFTLTISSLQPEDVATYYCAGYRGAHTDGDAFGGGTKVEIKGGGGSGGGGSGGGGSGGGGSEQQLVESGGGLVKPGGSLRLSCAASGFSFSRSSYMCWVRQAPGKGLEWIGCLSVGDGHTYYASWAKGRFTISKDSAKNSVYLQMNSLRAEDTAVYFCARAPSYSGDGGHGYDLWGPGTLVTVSS

SEQ ID NO: 245 - protein, 217 aa, synthetic construct
AVVMTQTPASVEAAVGGTVTINCQASQRINNYLSWFQQKPGQPPKLLIYGAATLASGVPSRFKGSGSGTEYTLTISDLEPADAATYYCQCTYGIPSSNYGFGGGTEVVVKRTVAAPSVFIFPPSDEQLKSGTASVVCLLNNFYPREAKVQWKVDNALQSGNSQESVTEQDSKDSTYSLSSTLTLSKADYEKHKVYACEVTHQGLSSPVTKSFNRGEC

SEQ ID NO: 246 - protein, 724 aa, synthetic construct
QSLEESGGDLVKPGGTLTLTCTASGFSFSSSYWLCWVRQAPGKGLEWIACIYGGSSRGTYYASWAKGRFTISKTSSTTVTLQMTSLTAADTATYFCASHTYTYPRFSPYFNLWGPGTLVSVSSASTKGPSVFPLAPSSKSTSGGTAALGCLVKDYFPEPVTVSWNSGALTSGVHTFPAVLQSSGLYSLSSVVTVPSSSLGTQTYICNVNHKPSNTKVDKKVEPKSCDKTHTCPPCPAPEAAGGPSVFLFPPKPKDTLMISRTPEVTCVVVDVSHEDPEVKFNWYVDGVEVHNAKTKPREEQYNSTYRVVSVLTVLHQDWLNGKEYKCKVSNKALGAPIEKTISKAKGQPREPQVYTLPPSRDELTKNQVSLTCLVKGFYPSDIAVEWESNGQPENNYKTTPPVLDSDGSFFLYSKLTVDKSRWQQGNVFSCSVMHEALHNHYTQKSLSLSPGKGGGGSGGGGSGGGGSDIQMTQSPSSLSASVGDRVTITCQASESVDRNNRLAWFQQKPGKPPKLLIYTTSTLASGVPSRFSGSGSGTDFTLTISSLQPEDVATYYCAGYRGAHTDGDAFGGGTKVEIKGGGGSGGGGSGGGGSGGGGSEQQLVESGGGLVKPGGSLRLSCAASGFSFSRSSYMCWVRQAPGKGLEWIGCLSVGDGHTYYASWAKGRFTISKDSAKNSVYLQMNSLRAEDTAVYFCARAPSYSGDGGHGYDLWGPGTLVTVSS

SEQ ID NO: 247 - protein, 217 aa, synthetic construct
AFEMTQTPASVSPAVGGTVSINCQASEDIESSLAWYQQKPGQPPKLLIYDASDLESGVPSRFKGSGSGTEYTLTISGVQPADAATYFCQSAYYTGSADNTFGGGTEVVVKRTVAAPSVFIFPPSDEQLKSGTASVVCLLNNFYPREAKVQWKVDNALQSGNSQESVTEQDSKDSTYSLSSTLTLSKADYEKHKVYACEVTHQGLSSPVTKSFNRGEC